European Patent Application EP 4 218 801 A2, published August 2, 2023. Title: ANTIBODY MODIFICATION METHOD FOR PURIFYING BISPECIFIC ANTIBODY. Applicant: Chugai Seiyaku Kabushiki Kaisha. The sequence listing filed with the application follows.

SEQUENCE LISTING (25 sequences)

SEQ ID NO: 1 - DNA, 354 bp, synthetic construct
  misc_feature 1..354: note = An artificially synthesized sequence
  source 1..354: mol_type = other DNA
caggtccagcttgtgcagtctggggctgaggtgaagaagcctgggtcctcagtgaaggtttcctgcaaggcctctggaggcaccttcagtgactactatatgcactgggtgcgccaggcccccggacaagggcttgagtggatgggatacattaatcctagcagtggttatactaagtacaatcggaagttcagggacagagtcaccattaccgcggacaaatccacgagcacagcctacatggagctgagcagcctgagatctgaagacacggctgtgtattactgtgcgagagggggtaacggttactaccttgactactggggccagggcaccacggtcaccgtctcctca

SEQ ID NO: 2 - protein, 118 aa, synthetic construct
  REGION 1..118: note = An artificially synthesized sequence
QVQLVQSGAEVKKPGSSVKVSCKASGGTFSDYYMHWVRQAPGQGLEWMGYINPSSGYTKYNRKFRDRVTITADKSTSTAYMELSSLRSEDTAVYYCARGGNGYYLDYWGQGTTVTVSS

SEQ ID NO: 3 - DNA, 357 bp, synthetic construct
  misc_feature 1..357: note = An artificially synthesized sequence
  source 1..357: mol_type = other DNA
caggtgcagctggtgcagtctggacctgacgtgaagaagccgggggcctcagtgaaggtctcctgcaaggcctctggctacatgttttccgacaacaacatggactgggcgcgacaggcccctggacaagggcttgagtggatgggagatattaatactaaaagtggtggttctatctacaaccagaagttcaagggcagagtcatcatgaccatagacaaatccacgggcacagcctacatggaattgaggagcctgagatcagacgacacggccatatattactgtgcgaggaggaggagctacggctactactttgactactggggccagggaaccctggtcaccgtctcctca

SEQ ID NO: 4 - protein, 119 aa, synthetic construct
  REGION 1..119: note = An artificially synthesized sequence
QVQLVQSGPDVKKPGASVKVSCKASGYMFSDNNMDWARQAPGQGLEWMGDINTKSGGSIYNQKFKGRVIMTIDKSTGTAYMELRSLRSDDTAIYYCARRRSYGYYFDYWGQGTLVTVSS

SEQ ID NO: 5 - DNA, 318 bp, synthetic construct
  misc_feature 1..318: note = An artificially synthesized sequence
  source 1..318: mol_type = other DNA
gacatcgtgatgacccagtctccatcctccctgtctgcatctgtaggagacagagtcaccatcacttgcaaggccagtcagaatgtggggactgctgtagcctggtatcagcagaaaccagggaaagcccctaagctcctgatctattcggcatcctaccggtacagtggggtcccatcaaggttcagtggcagtcgatatgggacagatttcactctcaccatctcaagcttgcaacctgaagatttagcaacttactactgtcagcaatatagcaactatatcacgttcggcggagggaccaaggtggagatcaaa

SEQ ID NO: 6 - protein, 106 aa, synthetic construct
  REGION 1..106: note = An artificially synthesized sequence
DIVMTQSPSSLSASVGDRVTITCKASQNVGTAVAWYQQKPGKAPKLLIYSASYRYSGVPSRFSGSRYGTDFTLTISSLQPEDLATYYCQQYSNYITFGGGTKVEIK

SEQ ID NO: 7 - protein, 118 aa, synthetic construct
  REGION 1..118: note = An artificially synthesized sequence
QVQLVQSGAEVKKPGSSVKVSCKASGGTFSDYYMHWVRQAPGEGLEWMGYINPSSGYTKYNRKFRDRVTITADKSTSTAYMELSSLRSEDTAVYYCARGGNGYYLDYWGEGTTVTVSS

SEQ ID NO: 8 - protein, 118 aa, synthetic construct
  REGION 1..118: note = An artificially synthesized sequence
QVQLVQSGAEVVKPGSSVKVSCKASGGTFSDYYMHWVRQAPGEGLEWMGYINPSSGYTKYNRKFRDRVTITADKSTSTAYMELSSLRSEDTAVYYCARGGNGYYLDYWGEGTTVTVSS

SEQ ID NO: 9 - protein, 118 aa, synthetic construct
  REGION 1..118: note = An artificially synthesized sequence
QVQLVQSGAEVKKPGSSVKVSCTASGGTFSDYYMHWVRQAPGEGLEWMGYINPSSGYTKYNRKFRDRVTITADKSTSTAYMELSSLRSEDTAVYYCARGGNGYYLDYWGEGTTVTVSS

SEQ ID NO: 10 - protein, 118 aa, synthetic construct
  REGION 1..118: note = An artificially synthesized sequence
QVQLVQSGAEVVKPGSSVKVSCTASGGTFSDYYMHWVRQAPGEGLEWMGYINPSSGYTKYNRKFRDRVTITADKSTSTAYMELSSLRSEDTAVYYCARGGNGYYLDYWGEGTTVTVSS

SEQ ID NO: 11 - protein, 118 aa, synthetic construct
  REGION 1..118: note = An artificially synthesized sequence
EVQLVQSGAEVVKPGSSVKVSCTASGYTFSDYYMHWVRQAPGEGLEWMGYINPSSGYTKYNRKFRDRVTITADKSTSTAYMELSSLRSEDTAVYYCARGGLGYYLDYWGEGTTVTVSS

SEQ ID NO: 12 - protein, 118 aa, synthetic construct
  REGION 1..118: note = An artificially synthesized sequence
EVQLVQSGAEVQKPGASVKVSCKASGYTFTDYYMHWVRQAPGEGLEWMGYINPSSGYTKYNRKFRDRVTITADKSTSTAYMELSSLRSEDTAVYYCARGGQGYYLDYWGEGTTVTVSS

SEQ ID NO: 13 - protein, 118 aa, synthetic construct
  REGION 1..118: note = An artificially synthesized sequence
QVQLVQSGAEVKKPGSSVKVSCKASGGTFSDYYMHWVRQAPGQGLEWMGYINPSSGYTKYNRKFRDRVTITADKSTSTAYMELSSLRSEDTAVYYCARGGRGYYLDYWGQGTTVTVSS

SEQ ID NO: 14 - protein, 119 aa, synthetic construct
  REGION 1..119: note = An artificially synthesized sequence
QVQLVQSGPDVKKPGASVKVSCKASGYMFSDNNMDWARQAPGKGLEWMGDINTKSGGSIYNQKFKGRVIMTIDKSTGTAYMELRSLRSDDTAIYYCARRRSYGYYFDYWGRGTLVTVSS

SEQ ID NO: 15 - protein, 119 aa, synthetic construct
  REGION 1..119: note = An artificially synthesized sequence
QVQLVQSGPDVKKPGASVKVSCKASGYMFSDNNMDWARKAPGKGLEWMGDINTKSGGSIYNQKFKGRVIMTIDKSTGTAYMELRSLRSDDTAIYYCARRRSYGYYFDYWGRGTLVTVSS

SEQ ID NO: 16 - protein, 119 aa, synthetic construct
  REGION 1..119: note = An artificially synthesized sequence
EVQLVQSGAQVKKPGASVKVSCKASGYTFSDNNMDWVRQAPGKGLEWMGDINTKSGGSIYNQKFKGRVIMTIDKSTGTAYMELRSLRSDDTAIYYCARRRSYGYYFDYWGRGTLVTVSS

SEQ ID NO: 17 - protein, 106 aa, synthetic construct
  REGION 1..106: note = An artificially synthesized sequence
DIVMTQSPSSLSASVGDRVTITCKASQNVGTAVAWYQQKPGKAPKLLIYSASYRYSGVPSRFSGSRYGTDFTLTISSLQPEDLATYYCQQYSNYITFGQGTKVEIK

SEQ ID NO: 18 - protein, 106 aa, synthetic construct
  REGION 1..106: note = An artificially synthesized sequence
DIVMTQSPSSLSASVGDRVTITCKASQNVGTAVAWYQQKPGKAPKLLIYSASYRASGVPSRFSGSRYGTDFTLTISSLQPEDLATYYCQQYSNYITFGQGTKVEIK

SEQ ID NO: 19 - protein, 119 aa, Mus musculus
MEVQLQQSGAELVKPGASVKLSCTASGFNIKDYYMHWIKQRPGQGLEWLGYINPSSGYTKYNRKFRDKATLTADKSSSTAYMQLTSLTYEDSAVYYCARGGNGYYLDYWGQGTTLTVSS

SEQ ID NO: 20 - protein, 120 aa, Mus musculus
MQVQLQQSGPELVKPGASVKISCKASGYTFTDNNMDWVKQSHGKGLEWIGDINTKSGGSIYNQKFKGKATLTIDKSSSTAYMELRSLTSEDTAVYYCARRRSYGYYFDYWGQGTTLTVSS

SEQ ID NO: 21 - protein, 107 aa, Homo sapiens
DIVMTQSHKFMSTSVGDRVSITCKASQNVGTAVAWYQQKPGQSPKLLIYSASYRYSGVPDRFTGSRYGTDFTLTISNVQSEDLADYLCQQYSNYITFGGGTKLELKR

SEQ ID NO: 22 - DNA, 24 bp, synthetic construct
  misc_feature 1..24: note = an artificially synthesized primer sequence
  source 1..24: mol_type = other DNA
caccgtctcctcagcctccaccaa

SEQ ID NO: 23 - DNA, 24 bp, synthetic construct
  misc_feature 1..24: note = an artificially synthesized primer sequence
  source 1..24: mol_type = other DNA
gtggcactcatttacccggagaca

SEQ ID NO: 24 - DNA, 981 bp, Homo sapiens
  source 1..981: mol_type = other DNA
gctagcaccaagggcccatcggtcttccccctggcgccctgctccaggagcacctccgagagcacagcggccctgggctgcctggtcaaggactacttccccgaaccggtgacggtgtcgtggaactcaggcgctctgaccagcggcgtgcacaccttcccggctgtcctacagtcctcaggactctactccctcagcagcgtggtgaccgtgccctccagcaacttcggcacccagacctacacctgcaacgtagatcacaagcccagcaacaccaaggtggacaagacagttgagcgcaaatgttgtgtcgagtgcccaccgtgcccagcaccacctgtggcaggaccgtcagtcttcctcttccccccaaaacccaaggacaccctcatgatctcccggacccctgaggtcacgtgcgtggtggtggacgtgagccacgaagaccccgaggtccagttcaactggtacgtggacggcgtggaggtgcataatgccaagacaaagccacgggaggagcagttcaacagcacgttccgtgtggtcagcgtcctcaccgtcgtgcaccaggactggctgaacggcaaggagtacaagtgcaaggtctccaacaaaggcctcccagcccccatcgagaaaaccatctccaaaaccaaagggcagccccgagaaccacaggtgtacaccctgcccccatcccgggaggagatgaccaagaaccaggtcagcctgacctgcctggtcaaaggcttctaccccagcgacatcgccgtggagtgggagagcaatgggcagccggagaacaactacaagaccacacctcccatgctggactccgacggctccttcttcctctacagcaagctcaccgtggacaagagcaggtggcagcaggggaacgtcttctcatgctccgtgatgcatgaggctctgcacaaccactacacacagaagagcctctccctgtctccgggtaaatga

SEQ ID NO: 25 - protein, 326 aa, Homo sapiens
ASTKGPSVFPLAPCSRSTSESTAALGCLVKDYFPEPVTVSWNSGALTSGVHTFPAVLQSSGLYSLSSVVTVPSSNFGTQTYTCNVDHKPSNTKVDKTVERKCCVECPPCPAPPVAGPSVFLFPPKPKDTLMISRTPEVTCVVVDVSHEDPEVQFNWYVDGVEVHNAKTKPREEQFNSTFRVVSVLTVVHQDWLNGKEYKCKVSNKGLPAPIEKTISKTKGQPREPQVYTLPPSREEMTKNQVSLTCLVKGFYPSDIAVEWESNGQPENNYKTTPPMLDSDGSFFLYSKLTVDKSRWQQGNVFSCSVMHEALHNHYTQKSLSLSPGK